European Patent Specification EP 3 910 068 B1, published January 28, 2026. Title: Molecular Tagging Methods and Sequencing Libraries. Applicant: Translational Genomics Research Institute. The sequence listing filed with the application follows.

SEQUENCE LISTING (4 sequences)

SEQ ID NO: 1 - DNA, 40 bp, Artificial Sequence
  Primer
cgctcttccgatctctgatccagacaactgttcaaactga

SEQ ID NO: 2 - DNA, 37 bp, Artificial Sequence
  Primer
gtgactggagttcagacgtgtgctcttccgatctgac

SEQ ID NO: 3 - DNA, 53 bp, Artificial Sequence
  Hairpin adapter
  misc_feature (10)..(18): n is any nucleotide
  misc_feature (36)..(41): n is any nucleotide
tgctctttgnnnnnnnnngtcagatcggaagagcannnnnnctgcccatagag

SEQ ID NO: 4 - DNA, 67 bp, Artificial Sequence
  barcode primer
caagcagaagacggcatacgagatcgtgatgtgactggagttcagacgtgtgctcttccgatctgac